European Patent Application EP 4 559 323 A2, published May 28, 2025. Title: NON-ANIMAL BASED PROTEIN SOURCES WITH FUNCTIONAL PROPERTIES. Applicant: Clara Foods Co. The sequence listing filed with the application follows.

SEQUENCE LISTING (75 sequences)

SEQ ID NO: 1 - protein, 474 aa, synthetic construct
  REGION 1..474: note = Synthetic Polypeptide
MRFPSIFTAVLFAASSALAAPVNTTTEDETAQIPAEAVIGYSDLEGDFDVAVLPFSNSTNNGLLFINTTIASIAAKEEGVSLDKREAEAGSIGAASMEFCFDVFKELKVHHANENIFYCPIAIMSALAMVYLGAKDSTRTQINKVVRFDKLPGFGDSIEAQCGTSVNVHSSLRDILNQITKPNDVYSFSLASRLYAEERYPILPEYLQCVKELYRGGLEPINFQTAADQARELINSWVESQTNGIIRNVLQPSSVDSQTAMVLVNAIVFKGLWEKAFKDEDTQAMPFRVTEQESKPVQMMYQIGLFRVASMASEKMKILELPFASGTMSMLVLLPDEVSGLEQLESIINFEKLTEWTSSNVMEERKIKVYLPRMKMEEKYNLTSVLMAMGITDVFSSSANLSGISSAESLKISQAVHAAHAEINEAGREVVGSAEAGVDAASVSEEFRADHPFLFCIKHIATNAVLFFGRCVSP

SEQ ID NO: 2 - protein, 389 aa, synthetic construct
  REGION 1..389: note = Synthetic Polypeptide
EAEAGSIGAASMEFCFDVFKELKVHHANENIFYCPIAIMSALAMVYLGAKDSTRTQINKVVRFDKLPGFGDSIEAQCGTSVNVHSSLRDILNQITKPNDVYSFSLASRLYAEERYPILPEYLQCVKELYRGGLEPINFQTAADQARELINSWVESQTNGIIRNVLQPSSVDSQTAMVLVNAIVFKGLWEKAFKDEDTQAMPFRVTEQESKPVQMMYQIGLFRVASMASEKMKILELPFASGTMSMLVLLPDEVSGLEQLESIINFEKLTEWTSSNVMEERKIKVYLPRMKMEEKYNLTSVLMAMGITDVFSSSANLSGISSAESLKISQAVHAAHAEINEAGREVVGSAEAGVDAASVSEEFRADHPFLFCIKHIATNAVLFFGRCVSP

SEQ ID NO: 3 - protein, 419 aa, synthetic construct
  REGION 1..419: note = Synthetic Polypeptide
MRVPAQLLGLLLLWLPGARCGSIGAASMEFCFDVFKELKVHHANENIFYCPIAIMSALAMVYLGAKDSTRTQINKVVRFDKLPGFGDSIEAQCGTSVNVHSSLRDILNQITKPNDVYSFSLASRLYAEERYPILPEYLQCVKELYRGGLEPINFQTAADQARELINSWVESQTNGIIRNVLQPSSVDSQTAMVLVNAIVFKGLWEKAFKDEDTQAMPFRVTEQESKPVQMMYQIGLFRVASMASEKMKILELPFASGTMSMLVLLPDEVSGLEQLESIINFEKLTEWTSSNVMEERKIKVYLPRMKMEEKYNLTSVLMAMGITDVFSSSANLSGISSAESLKISQAVHAAHAEINEAGREVVGSAEAGVDAASVSEEFRADHPFLFCIKHIATNAVLFFGRCVSPLEIKRAAAHHHHHH

SEQ ID NO: 4 - protein, 406 aa, synthetic construct
  REGION 1..406: note = Synthetic Polypeptide
MTSGFANELGPRLMGKLTMGSIGAASMEFCFDVFKELKVHHANENIFYCPIAIMSALAMVYLGAKDSTRTQINKVVRFDKLPGFGDSIEAQCGTSVNVHSSLRDILNQITKPNDVYSFSLASRLYAEERYPILPEYLQCVKELYRGGLEPINFQTAADQARELINSWVESQTNGIIRNVLQPSSVDSQTAMVLVNAIVFKGLWEKTFKDEDTQAMPFRVTEQESKPVQMMYQIGLFRVASMASEKMKILELPFASGTMSMLVLLPDEVSGLEQLESIINFEKLTEWTSSNVMEERKIKVYLPRMKMEEKYNLTSVLMAMGITDVFSSSANLSGISSAESLKISQAVHAAHAEINEAGREVVGSAEAGVDAASVSEEFRADHPFLFCIKHIATNAVLFFGRCVSPSR

SEQ ID NO: 5 - protein, 451 aa, synthetic construct
  REGION 1..451: note = Synthetic Polypeptide
MGGRRVRWEVYISRAGYVNRQIAWRRHHRSLTMRVPAQLLGLLLLWLPGARCGSIGAASMEFCFDVFKELKVHHANENIFYCPIAIMSALAMVYLGAKDSTRTQINKVVRFDKLPGFGDSIEAQCGTSVNVHSSLRDILNQITKPNDVYSFSLASRLYAEERYPILPEYLQCVKELYRGGLEPINFQTAADQARELINSWVESQTNGIIRNVLQPSSVDSQTAMVLVNAIVFKGLWEKAFKDEDTQAMPFRVTEQESKPVQMMYQIGLFRVASMASEKMKILELPFASGTMSMLVLLPDEVSGLEQLESIINFEKLTEWTSSNVMEERKIKVYLPRMKMEEKYNLTSVLMAMGITDVFSSSANLSGISSAESLKISQAVHAAHAEINEAGREVVGSAEAGVDAASVSEEFRADHPFLFCIKHIATNAVLFFGRCVSPLEIKRAAAHHHHHH

SEQ ID NO: 6 - protein, 386 aa, synthetic construct
  REGION 1..386: note = Synthetic Polypeptide
MGSIGAVSMEFCFDVFKELKVHHANENIFYSPFTIISALAMVYLGAKDSTRTQINKVVRFDKLPGFGDSVEAQCGTSVNVHSSLRDILNQITKPNDVYSFSLASRLYAEETYPILPEYLQCVKELYRGGLESINFQTAADQARGLINSWVESQTNGMIKNVLQPSSVDSQTAMVLVNAIVFKGLWEKAFKDEDTQAIPFRVTEQESKPVQMMYQIGLFKVASMASEKMKILELPFASGTMSMWVLLPDEVSGLEQLETTISFEKMTEWISSNIMEERRIKVYLPRMKMEEKYNLTSVLMAMGITDLFSSSANLSGISSAGSLKISQAVHAAYAEIYEAGREVIGSAEAGADATSVSEEFRVDHPFLYCIKHNLTNSILFFGRCISP

SEQ ID NO: 7 - protein, 386 aa, synthetic construct
  REGION 1..386: note = Synthetic Polypeptide
MGSIGAVSMEFCFDVFKELKVHHANENIFYSPFTIISALAMVYLGAKDSTRTQINKVVRFDKLPGFGDSVEAQCGTSVNVHSSLRDILNQITKPNDVYSFSLASRLYAEETYPILPEYLQCVKELYRGGLESINFQTAADQARGLINSWVESQTNGMIKNVLQPSSVDSQTAMVLVNAIVFKGLWEKAFKDEDTQAIPFRVTEQESKPVQMMYQIGLFKVASMASEKMKILELPFASGTMSMWVLLPDEVSGLEQLETTISFEKMTEWISSNIMEERRIKVYLPRMKMEEKYNLTSVLMAMGITDLFSSSANLSGISSAGSLKISQAAHAAYAEIYEAGREVIGSAEAGADATSVSEEFRVDHPFLYCIKHNLTNSILFFGRCISP

SEQ ID NO: 8 - protein, 417 aa, synthetic construct
  REGION 1..417: note = Synthetic Polypeptide
YYRVPCMVLCTAFHPYIFIVLLFALDNSEFTMGSIGAVSMEFCFDVFKELRVHHPNENIFFCPFAIMSAMAMVYLGAKDSTRTQINKVIRFDKLPGFGDSTEAQCGKSANVHSSLKDILNQITKPNDVYSFSLASRLYADETYSIQSEYLQCVNELYRGGLESINFQTAADQARELINSWVESQTNGIIRNVLQPSSVDSQTAMVLVNAIVFRGLWEKAFKDEDTQTMPFRVTEQESKPVQMMYQIGSFKVASMASEKMKILELPLASGTMSMLVLLPDEVSGLEQLETTISFEKLTEWTSSNVMEERKIKVYLPRMKMEEKYNLTSVLMAMGITDLFRSSANLSGISLAGNLKISQAVHAAHAEINEAGRKAVSSAEAGVDATSVSEEFRADRPFLFCIKHIATKVVFFFGRYTSP

SEQ ID NO: 9 - protein, 383 aa, synthetic construct
  REGION 1..383: note = Synthetic Polypeptide
MGSIGAASMEFCFDVFKELKVHHANDNMLYSPFAILSTLAMVFLGAKDSTRTQINKVVHFDKLPGFGDSIEAQCGTSVNVHSSLRDILNQITKQNDAYSFSLASRLYAQETYTVVPEYLQCVKELYRGGLESVNFQTAADQARGLINAWVESQTNGIIRNILQPSSVDSQTAMVLVNAIAFKGLWEKAFKAEDTQTIPFRVTEQESKPVQMMYQIGSFKVASMASEKMKILELPFASGTMSMLVLLPDDVSGLEQLESIISFEKLTEWTSSSIMEERKVKVYLPRMKMEEKYNLTSLLMAMGITDLFSSSANLSGISSVGSLKISQAVHAAHAEINEAGRDVVGSAEAGVDATEEFRADHPFLFCVKHIETNAILLFGRCVSP

SEQ ID NO: 10 - protein, 386 aa, synthetic construct
  REGION 1..386: note = Synthetic Polypeptide
MASIGAVSTEFCVDVYKELRVHHANENIFYSPFTIISTLAMVYLGAKDSTRTQINKVVRFDKLPGFGDSIEAQCGTSVNVHSSLRDILNQITKPNDVYSFSLASRLYAEETYPILPEYLQCVKELYRGGLESINFQTAADQARELINSWVESQTSGIIKNVLQPSSVNSQTAMVLVNAIYFKGLWERAFKDEDTQAIPFRVTEQESKPVQMMSQIGSFKVASVASEKVKILELPFVSGTMSMLVLLPDEVSGLEQLESTISTEKLTEWTSSSIMEERKIKVFLPRMRMEEKYNLTSVLMAMGMTDLFSSSANLSGISSAESLKISQAVHAAYAEIYEAGREVVSSAEAGVDATSVSEEFRVDHPFLLCIKHNPTNSILFFGRCISP

SEQ ID NO: 11 - protein, 411 aa, synthetic construct
  REGION 1..411: note = Synthetic Polypeptide
MALCKAFHPYIFIVLLFDVDNSAFTMASIGAVSTEFCVDVYKELRVHHANENIFYSPFTIISTLAMVYLGAKDSTRTQINKVVRFDKLPGFGDSIEAQCGTSVNVHSSLRDILNQITKPNDVYSFSLASRLYAEETYPILPEYLQCVKELYRGGLESINFQTAADQARELINSWVESQTSGIIKNVLQPSSVNSQTAMVLVNAIYFKGLWERAFKDEDTQAIPFRVTEQESKPVQMMSQIGSFKVASVASEKVKILELPFVSGTMSMLVLLPDEVSGLEQLESTISTEKLTEWTSSSIMEERKIKVFLPRMRMEEKYNLTSVLMAMGMTDLFSSSANLSGISSAESLKISQAVHAAYAEIYEAGREVVSSAEAGVDATSVSEEFRVDHPFLLCIKHNPTNSILFFGRCISP

SEQ ID NO: 12 - protein, 383 aa, synthetic construct
  REGION 1..383: note = Synthetic Polypeptide
MGSIGAASMEFCFDVFKELKVHHANDNMLYSPFAILSTLAMVFLGAKDSTRTQINKVVHFDKLPGFGDSIEAQCGTSANVHSSLRDILNQITKQNDAYSFSLASRLYAQETYTVVPEYLQCVKELYRGGLESVNFQTAADQARGLINAWVESQTNGIIRNILQPSSVDSQTAMVLVNAIAFKGLWEKAFKAEDTQTIPFRVTEQESKPVQMMHQIGSFKVASMASEKMKILELPFASGTMSMLVLLPDDVSGLEQLESTISFEKLTEWTSSSIMEERKVKVYLPRMKMEEKYNLTSLLMAMGITDLFSSSANLSGISSVGSLKISQAVHAAYAEINEAGRDVVGSAEAGVDATEEFRADHPFLFCVKHIETNAILLFGRCVSP

SEQ ID NO: 13 - protein, 408 aa, synthetic construct
  REGION 1..408: note = Synthetic Polypeptide
MGLCTAFHPYIFIVLLFALDNSEFTMGSIGAASMEFCFDVFKELKVHHANDNMLYSPFAILSTLAMVFLGAKDSTRTQINKVVHFDKLPGFGDSIEAQCGTSANVHSSLRDILNQITKQNDAYSFSLASRLYAQETYTVVPEYLQCVKELYRGGLESVNFQTAADQARGLINAWVESQTNGIIRNILQPSSVDSQTAMVLVNAIAFKGLWEKAFKAEDTQTIPFRVTEQESKPVQMMHQIGSFKVASMASEKMKILELPFASGTMSMLVLLPDDVSGLEQLESTISFEKLTEWTSSSIMEERKVKVYLPRMKMEEKYNLTSLLMAMGITDLFSSSANLSGISSVGSLKISQAVHAAYAEINEAGRDVVGSAEAGVDATEEFRADHPFLFCVKHIETNAILLFGRCVSP

SEQ ID NO: 14 - protein, 383 aa, synthetic construct
  REGION 1..383: note = Synthetic Polypeptide
MGSIGAASMEFCFDVFKELKVHHANDNMLYSPFAILSTLAMVFLGAKDSTRTQINKVVHFDKLPGFGDSIEAQCGTSANVHSSLRDILNQITKQNDAYSFSLASRLYAQETYTVVPEYLQCVKELYRGGLESVNFQTAADQARGLINAWVESQTNGIIRNILQPSSVDSQTAMVLVNAIAFKGLWEKAFKAEDTQTIPFRVTEQESKPVQMMHQIGSFKVASMASEKMKILELPFASGTMSMLVLLPDDVSGLEQLESTISFEKLTEWTSSSIMEERKVKVYLPRMKMEEKYNLTSLLMAMGITDLFSSSANLSGISSVGSLKIPQAVHAAYAEINEAGRDVVGSAEAGVDATEEFRADHPFLFCVKHIETNAILLFGRCVSP

SEQ ID NO: 15 - protein, 386 aa, synthetic construct
  REGION 1..386: note = Synthetic Polypeptide
MGSIGAASTEFCFDVFRELRVQHVNENIFYSPFSIISALAMVYLGARDNTRTQIDKVVHFDKLPGFGESMEAQCGTSVSVHSSLRDILTQITKPSDNFSLSFASRLYAEETYAILPEYLQCVKELYKGGLESISFQTAADQARELINSWVESQTNGIIKNILQPSSVDSQTTMVLVNAIYFKGMWEKAFKDEDTQAMPFRMTEQESKPVQMMYQVGSFKVAMVTSEKMKILELPFASGMMSMFVLLPDEVSGLEQLESTISFEKLTEWTSSTMMEERRMKVYLPRMKMEEKYNLTSVFMALGMTDLFSSSANMSGISSTVSLKMSEAVHAACVEIFEAGRDVVGSAEAGMDVTSVSEEFRADHPFLFFIKHNPTNSILFFGRWMSP

SEQ ID NO: 16 - protein, 386 aa, synthetic construct
  REGION 1..386: note = Synthetic Polypeptide
MGSIGAASTEFCFDVFRELKVQHVNENIFYSPLSIISALAMVYLGARDNTRTQIDQVVHFDKIPGFGESMEAQCGTSVSVHSSLRDILTEITKPSDNFSLSFASRLYAEETYTILPEYLQCVKELYKGGLESISFQTAADQARELINSWVESQTNGIIKNILQPSSVDSQTTMVLVNAIYFKGMWEKAFKDEDTQTMPFRMTEQESKPVQMMYQVGSFKLATVTSEKVKILELPFASGMMSMCVLLPDEVSGLEQLETTISFEKLTEWTSSTMMEERRMKVYLPRMKMEEKYNLTSVFMALGMTDLFSSSANMSGISSTVSLKMSEAVHAACVEIFEAGRDVVGSAEAGMDVTSVSEEFRADHPFLFFIKHNPSNSILFFGRWISP

SEQ ID NO: 17 - protein, 386 aa, synthetic construct
  REGION 1..386: note = Synthetic Polypeptide
MGSIGAASTEFCFDVFKELKVQHVNENIFYSPLTIISALSMVYLGARENTRAQIDKVLHFDKMPGFGDTIESQCGTSVSIHTSLKDMFTQITKPSDNYSLSFASRLYAEETYPILPEYLQCVKELYKGGLETISFQTAAEQARELINSWVESQTNGMIKNILQPSSVDPQTKMVLVNAIYFKGVWEKAFKDEDTQEVPFRVTEQESKPVQMMYQIGSFKVAVMASEKMKILELPYASGQLSMLVLLPDDVSGLEQLESAITFEKLMAWTSSTTMEERKMKVYLPRMKIEEKYNLTSVLMALGVTDLFSSSANLSGISSAESLKISKAVHEAFVEIYEAGSEVVGSTEAGMEVTSVSEEFRADHPFLFLIKHNPTNSILFFGRCFSP

SEQ ID NO: 18 - protein, 386 aa, synthetic construct
  REGION 1..386: note = Synthetic Polypeptide
MGSIGAASTEFCFDVFKELKVQHVNENIFYSPLTIISALSMVYLGARENTRTQIDKVLHFDKMTGFGDTVESQCGTSVSIHTSLKDIFTQITKPSDNYSLSLASRLYAEETYPILPEYLQCVKELYKGGLETVSFQTAAEQARELINSWVESQTNGMIKNILQPSSVDPQTKMVLVNAIYFKGVWEKAFKDEDTQEVPFRVTEQESKPVQMMYQIGSFKVAVMASEKMKILELPYASGQLSMLVLLPDDVSGLEQLESAITSEKLMEWTSSTTMEERKMKVYLPRMKIEEKYNLTSVLMALGVTDLFSSSADLSGISSAESLKISKAVHEAFVEIYEAGSEVVGSTEGGMEVTSVSEEFRADHPFLFLIKHKPTNSILFFGRCFSP

SEQ ID NO: 19 - protein, 386 aa, synthetic construct
  REGION 1..386: note = Synthetic Polypeptide
MGSIGAASTEFCFDVFKELKVQHVNENIFYSPLTIISALSMVYLGARENTRTQIDKVLHFDKMTGFGDTVESQCGTSVSIHTSLKDIFTQITKPSDNYSLSLASRLYAEETYPILPEYLQCVKELYKGGLETVSFQTAAEQARELINSWVESQTNGMIKNILQPSSVDPQTKMVLVNAIYFKGVWEKAFKDEDTQEVPFRVTEQESKPVQMMYQIGSFKVAVMASEKMKILELPYASGQLSMLVLLPDDVSGLEQLESAITSEKLMEWTSSTTMEERKMKVYLPRMKIEEKYNLTSVLMALGVTDLFSSSADLSGISSAESLKISKAVHEAFVEIYEAGSEVVGSTEGGMEVTSFSEEFRADHPFLFLIKHKPTNSILFFGRCFSP

SEQ ID NO: 20 - protein, 386 aa, synthetic construct
  REGION 1..386: note = Synthetic Polypeptide
MGSIGAASTEFCFDVFKELKVQHVNENIFYSPLSIISALSMVYLGARENTRAQIDKVVHFDKITGFGETIESQCGTSVSVHTSLKDMFTQITKPSDNYSLSFASRLYAEETYPILPEYLQCVKELYKGGLETTSFQTAADQARELINSWVESQTNGMIKNILQPGSVDPQTEMVLVNAIYFKGMWEKAFKDEDTQAVPFRMTEQESKTVQMMYQIGSFKVAVMASEKMKILELPYASGELSMLVMLPDDVSGLEQLETAITFEKLMEWTSSNMMEERKMKVYLPRMKMEEKYNLTSVLMALGVTDLFSSSANLSGISSAESLKMSEAVHEAFVEIYEAGSEVVGSTGAGMEVTSVSEEFRADHPFLFLIKHNPTNSILFFGRCFSP

SEQ ID NO: 21 - protein, 386 aa, synthetic construct
  REGION 1..386: note = Synthetic Polypeptide
MGSIGAASTEFCFDVFKELRVQHVNENVCYSPLIIISALSLVYLGARENTRAQIDKVVHFDKITGFGESIESQCGTSVSVHTSLKDMFNQITKPSDNYSLSVASRLYAEERYPILPEYLQCVKELYKGGLESISFQTAADQAREAINSWVESQTNGMIKNILQPSSVDPQTEMVLVNAIYFKGMWQKAFKDEDTQAVPFRISEQESKPVQMMYQIGSFKVAVMAAEKMKILELPYASGELSMLVLLPDEVSGLEQLENAITVEKLMEWTSSSPMEERIMKVYLPRMKIEEKYNLTSVLMALGITDLFSSSANLSGISAEESLKMSEAVHQAFAEISEAGSEVVGSSEAGIDATSVSEEFRADHPFLFLIKHNATNSILFFGRCFSP

SEQ ID NO: 22 - protein, 386 aa, synthetic construct
  REGION 1..386: note = Synthetic Polypeptide
MGSISAASTEFCFDVFKELKVQHVNENIFYSPLSIISALSMVYLGARENTRAQIEKVVHFDKITGFGESIESQCSTSVSVHTSLKDMFTQITKPSDNYSLSFASRFYAEETYPILPEYLQCVKELYKGGLETINFRTAADQARELINSWVESQTNGMIKNILQPGSVDPQTDMVLVNAIYFKGMWEKAFKDEDTQALPFRVTEQESKPVQMMYQIGSFKVAVLASEKVKILELPYASGQLSMLVLLPDDVSGLEQLETAITVEKLMEWTSSNNMEERKIKVYLPRIKIEEKYNLTSVLMALGITDLFSSSANLSGISSAESLKVSEAIHEAFVEIYEAGSEVAGSTEAGIEVTSVSEEFRADHPFLFLIKHNATNSILFFGRCFSP

SEQ ID NO: 23 - protein, 386 aa, synthetic construct
  REGION 1..386: note = Synthetic Polypeptide
MVSIGAASTEFCFDVFKELKVQHVNENIFYSPLSIISALSMVYLGARENTRAQIDKVVHFDKITGFEETIESQCSTSVSVHTSLKDMFTQITKPSDNYSLSFASRLYAEETYPILPEYLQCVKELYKGGLETISFQTAADQARELINSWVESQTDGMIKNILQPGSVDPQTEMVLVNAIYFKGMWEKAFKDEDTQAVPFRMTEQESKPVQMMYQIGSFKVAVMASEKMKILELPYASGGMSMLVMLPDDVSGLEQLETAITFEKLMEWTSSNMMEERKMKVYLPRMKMEEKYNLTSVLMALGMTDLFSSSANLSGISSAESLKMSEAVHEAFVEIYEAGSEAVGSTGAGMEVTSVSEEFRADHPFLFLIKHNPTNSILFFGRCFSP

SEQ ID NO: 24 - protein, 386 aa, synthetic construct
  REGION 1..386: note = Synthetic Polypeptide
MGSIGAASTEFCFDVFKELKVQHVNENIFYSPLSIISALSMVYLGARENTRAQIDKVVHFDKITGFGEPIESQCGISVSVHTSLKDMITQITKPSDNYSLSFASRLYAEETYPILPEYLQCVKELYKGGLETISFQTAADQARELINSWVENQTNGMIKNILQPGSVDPQTEMVLVNAVYFKGMWEKAFKDEDTQAVPFRMTEQESKPVQMMYQIGSFKVAVMASEKIKILELPYASGELSMLVLLPDDVSGLEQLETAITLDKLTEWTSSNAMEERKMKVYLPRMKIEKKYNLTSVLIALGMTDLFSSSANLSGISSAESLKMSEAIHEAFLEIYEAGSEVVGSTEAGMEVTSVSEEFRADHPFLFLIKHNPTNSILFFGRCLSP

SEQ ID NO: 25 - protein, 386 aa, synthetic construct
  REGION 1..386: note = Synthetic Polypeptide
MGSIGAASTEFCFDVFKELKVQHVNENIFYSPLTIISALSMVYLGARENTRAQIDKVVHFDKIPGFGDTTESQCGTSVSVHTSLKDMFTQITKPSDNYSVSFASRLYAEETYPILPEFLECVKELYKGGLESISFQTAADQARELINSWVESQTNGMIKNILQPGSVDSQTEMVLVNAIYFKGMWEKAFKDEDTQTVPFRMTEQETKPVQMMYQIGTFKVAVMPSEKMKILELPYASGELCMLVMLPDDVSGLEELESSITVEKLMEWTSSNMMEERKMKVFLPRMKIEEKYNLTSVLMALGMTDLFSSSANLSGISSAEPLKMSEAVHEAFIEIYEAGSEVVGSTGAGMEITSVSEEFRADHPFLFLIKHNPTNSILFFGRCVSP

SEQ ID NO: 26 - protein, 386 aa, synthetic construct
  REGION 1..386: note = Synthetic Polypeptide
MGSIGAVSTEFCFDVFKELKVQHVNENIFYSPLSIISALSMVYLGARENTRAQIDKVVHFDKITGSGETIEAQCGTSVSVHTSLKDMFTQITKPSENYSVGFASRLYADETYPIIPEYLQCVKELYKGGLEMISFQTAADQARELINSWVESQTNGMIKNILQPGSVDPQTEMILVNAIYFKGVWEKAFKDEDTQAVPFRMTEQESKPVQMMYQFGSFKVAAMAAEKMKILELPYASGALSMLVLLPDDVSGLEQLESAITFEKLMEWTSSNMMEEKKIKVYLPRMKMEEKYNFTSVLMALGMTDLFSSSANLSGISSADSLKMSEVVHEAFVEIYEAGSEVVGSTGSGMEAASVSEEFRADHPFLFLIKHNPTNSILFFGRCFSP

SEQ ID NO: 27 - protein, 391 aa, synthetic construct
  REGION 1..391: note = Synthetic Polypeptide
MVSIGAASTEFCFDVFKELKVQHVNENIFYSPLSIISALSMVYLGARENTRAQIDKVVHFDKITGFEETIESQVQKKQCSTSVSVHTSLKDMFTQITKPSDNYSLSFASRLYAEETYPILPEYLQCVKELYKGGLETISFQTAADQARELINSWVESQTDGMIKNILQPGSVDPQTEMVLVNAIYFKGMWEKAFKDEDTQAVPFRMTEQESKPVQMMYQIGSFKVAVMASEKMKILELPYASGGMSMLVMLPDDVSGLEQLETAITFEKLMEWTSSNMMEERKMKVYLPRMKMEEKYNLTSVLMALGMTDLFSSSANLSGISSAESLKMSEAVHEAFVEIYEAGSEAVGSTGAGMEVTSVSEEFRADHPFLFLIKHNPTNSILFFGRCFSP

SEQ ID NO: 28 - protein, 386 aa, synthetic construct
  REGION 1..386: note = Synthetic Polypeptide
MGSIGAASGEFCFDVFKELKVQHVNENIFYSPLSIISALSMVYLGARENTRAQIDKVVHFDKIIGFGESIESQCGTSVSVHTSLKDMFAQITKPSDNYSLSFASRLYAEETFPILPEYLQCVKELYKGGLETLSFQTAADQARELINSWVESQTNGMIKDILQPGSVDPQTEMVLVNAIYFKGVWEKAFKDEDTQTVPFRMTEQESKPVQMMYQIGSFKVAVVAAEKIKILELPYASGALSMLVLLPDDVSSLEQLETAITFEKLTEWTSSNIMEERKIKVYLPRMKIEEKYNLTSVLMDLGITDLFSSSANLSGISSAESLKVSEAIHEAIVDIYEAGSEVVGSSGAGLEGTSVSEEFRADHPFLFLIKHNPTSSILFFGRCFSP

SEQ ID NO: 29 - protein, 386 aa, synthetic construct
  REGION 1..386: note = Synthetic Polypeptide
MGSIGAASTEFCFDVFKELKVQHVNENIFYSPLSIISALSMVYLGARENTRAQIDKVVHFDKITGSGEAIESQCGTSVSVHISLKDMFTQITKPSDNYSLSFASRLYAEETYPILPEYLQCVKELYKEGLATISFQTAADQAREFINSWVESQTNGMIKNILQPGSVDPQTQMVLVNAIYFKGVWEKAFKDEDTQAVPFRMTKQESKPVQMMYQIGSFKVAVMASEKMKILELPYASGQLSMLVMLPDDVSGLEQIENAITFEKLMEWTNPNMMEERKMKVYLPRMKMEEKYNLTSVLMALGMTDLFSSSANLSGISSAESLKMSEAVHEAFVEIYEAGSEVVGSTGAGIEVTSVSEEFRADHPFLFLIKHNPTNSILFFGRCFSP

SEQ ID NO: 30 - protein, 386 aa, synthetic construct
  REGION 1..386: note = Synthetic Polypeptide
MGSIGEASTEFCIDVFRELKVQHVNENIFYSPLSIISALSMVYLGARENTRAQIDQVVHFDKITGFGDTVESQCGSSLSVHSSLKDIFAQITQPKDNYSLNFASRLYAEETYPILPEYLQCVKELYKGGLETISFQTAADQARELINSWVESQTNGMIKNILQPSSVDPQTEMVLVNAIYFKGVWEKAFKDEETQAVPFRITEQENRPVQIMYQFGSFKVAVVASEKIKILELPYASGQLSMLVLLPDEVSGLEQLENAITFEKLTEWTSSDIMEEKKIKVFLPRMKIEEKYNLTSVLVALGIADLFSSSANLSGISSAESLKMSEAVHEAFVEIYEAGSEVVGSSGAGIEAASDSEEFRADHPFLFLIKHKPTNSILFFGRCFSP

SEQ ID NO: 31 - protein, 386 aa, synthetic construct
  REGION 1..386: note = Synthetic Polypeptide
MGSIGAASTEFCFDIFNELKVQHVNENIFYSPLSIISALSMVYLGARENTKAQIDKVVHFDKITGFGESIESQCSTSASVHTSFKDMFTQITKPSDNYSLSFASRLYAEETYPILPEYSQCVKELYKGGLESISFQTAADQARELINSWVESQTNGMIKNILQPGSVDPQTELVLVNAIYFKGTWEKAFKDKDTQAVPFRVTEQESKPVQMMYQIGSYKVAVIASEKMKILELPYASGELSMLVLLPDDVSGLEQLETAITFEKLMEWTSSNMMEERKVKVYLPRMKIEEKYNLTSVLMALGMTDLFSPSANLSGISSAESLKMSEAIHEAFVEIYEAGSEVVGSTEAGMEVTSVSEEFRADHPFLFLIKCNLTNSILFFGRCFSP

SEQ ID NO: 32 - protein, 385 aa, synthetic construct
  REGION 1..385: note = Synthetic Polypeptide
MGSISTASTEFCFDVFKELKVQHVNENIFYSPLSIISALSMVYLGARENTRAQIEKVVHFDKITGFGESIESQCGTSVSVHTSLKDMLIQISKPSDNYSLSFASKLYAEETYPILPEYLQCVKELYKGGLESINFQTAADQARQLINSWVESQTNGMIKDILQPSSVDPQTEMVLVNAIYFKGIWEKAFKDEDTQEVPFRITEQESKPVQMMYQIGSFKVAVIASEKIKILELPYASGELSMLIVLPDDVSGLEQLETAITFEKLIEWTSPSIMEERKTKVYLPRMKIEEKYNLTSVLMALGMTDLFSPSANLSGISSAESLKMSEAIHEAFVEIYEAGSEVVGSAEAGMEATSVSEFRVDHPFLFLIKHNPANIILFFGRCVSP

SEQ ID NO: 33 - protein, 386 aa, synthetic construct
  REGION 1..386: note = Synthetic Polypeptide
MGSIGAASTEFCFDVFKELKVQHVNENIFYSPLTIISALSLVYLGARENTRAQIDKVFHFDKISGFGETTESQCGTSVSVHTSLKEMFTQITKPSDNYSVSFASRLYAEDTYPILPEYLQCVKELYKGGLETISFQTAADQAREVINSWVESQTNGMIKNILQPGSVDSQTEMVLVNAIYFKGMWEKAFKDEDTQTMPFRITEQERKPVQMMYQAGSFKVAVMASEKMKILELPYASGEFCMLIMLPDDVSGLEQLENSFSFEKLMEWTTSNMMEERKMKVYIPRMKMEEKYNLTSVLMALGMTDLFSSSANLSGISSAETLKMSEAVHEAFMEIYEAGSEVVGSTGSGAEVTGVYEEFRADHPFLFLVKHKPTNSILFFGRCVSP

SEQ ID NO: 34 - protein, 386 aa, synthetic construct
  REGION 1..386: note = Synthetic Polypeptide
MGSIGAASTEFCFDIFNELKVQHVNENIFYSPLSIISALSMVYLGARENTKAQIDKVVHFDKITGFGETIESQCSTSVSVHTSLKDTFTQITKPSDNYSLSFASRLYAEETYPILPEYSQCVKELYKGGLETISFQTAADQARELINSWVESQTNGMIKNILQPGSVDPQTELVLVNAIYFKGTWEKAFKDKDTQAVPFRVTEQESKPVQMMYQIGSYKVAVIASEKMKILELPYASRELSMLVLLPDDVSGLEQLETAITFEKLMEWTSSNMMEERKVKVYLPRMKIEEKYNLTSVLMALGMTDLFSPSANLSGISSAESLKMSEAVHEAFVEIYEAGSEVVGSTGAGMEVTSVSEEFRADHPFLFLIKCNPTNSILFFGRCFSP

SEQ ID NO: 35 - protein, 386 aa, synthetic construct
  REGION 1..386: note = Synthetic Polypeptide
MGSISAASAEFCLDVFKELKVQHVNENIFYSPLSIISALSMVYLGARENTRAQIDKVVHFDKITGSGETIEFQCGTSANIHPSLKDMFTQITRLSDNYSLSFASRLYAEERYPILPEYLQCVKELYKGGLETISFQTAADQARELINSWVESQTNGMIKNILQPGSVNPQTEMVLVNAIYFKGLWEKAFKDEDTQTVPFRMTEQESKPVQMMYQVGSFKVAVMASDKIKILELPYASGELSMLVLLPDDVTGLEQLETSITFEKLMEWTSSNVMEERTMKVYLPHMRMEEKYNLTSVLMALGVTDLFSSSANLSGISSAESLKMSEAVHEAFVEIYESGSQVVGSTGAGTEVTSVSEEFRVDHPFLFLIKHNPTNSILFFGRCFSP

SEQ ID NO: 36 - protein, 385 aa, synthetic construct
  REGION 1..385: note = Synthetic Polypeptide
MGSIGAASVEFCFDVFKELKVQHVNENIFYSPLSIISALSMVYLGARENTKAQIDKVVHFDKIAGFGEAIESQCVTSASIHSLKDMFTQITKPSDNYSLSFASRLYAEEAYSILPEYLQCVKELYKGGLETISFQTAADQARDLINSWVESQTNGMIKNILQPGAVDLETEMVLVNAIYFKGMWEKAFKDEDTQTVPFRMTEQESKPVQMMYQVGSFKVAVMASDKIKILELPYASGQLSMVVVLPDDVSGLEQLEASITSEKLMEWTSSSIMEEKKIKVYFPHMKIEEKYNLTSVLMALGMTDLFSSSANLSGISSAEKLKVSEAVHEAFVEISEAGSEVVGSTEAGTEVTSVSEEFKADHPFLFLIKHNPTNSILFFGRCFSP

SEQ ID NO: 37 - protein, 386 aa, synthetic construct
  REGION 1..386: note = Synthetic Polypeptide
MGSIGAASSEFCFDIFKELKVQHVNENIFYSPLSIISALSMVYLGARENTRAQIDKVVPFDKITASGESIESQCSTSVSVHTSLKDIFTQITKSSDNHSLSFASRLYAEETYPILPEYLQCVKELYEGGLETISFQTAADQARELINSWIESQTNGRIKNILQPGSVDPQTEMVLVNAIYFKGMWEKAFKDEDTQAVPFRMTEQESKPVQVMHQIGSFKVAVLASEKIKILELPYASGELSMLVLLPDDVSGLEQLETAITFEKLMEWTSPNIMEERKIKVFLPRMKIEEKYNLTSVLMALGITDLFSPLANLSGISSAESLKMSEAIHEAFVEISEAGSEVIGSTEAEVEVTNDPEEFRADHPFLFLIKHNPTNSILFFGRCFSP

SEQ ID NO: 38 - protein, 386 aa, synthetic construct
  REGION 1..386: note = Synthetic Polypeptide
MGSIGAASTEFCFDVFKELKAQYVNENIFYSPMTIITALSMVYLGSKENTRAQIAKVAHFDKITGFGESIESQCGASASIQFSLKDLFTQITKPSGNHSLSVASRIYAEETYPILPEYLECMKELYKGGLETINFQTAANQARELINSWVERQTSGMIKNILQPSSVDSQTEMVLVNAIYFRGLWEKAFKVEDTQATPFRITEQESKPVQMMHQIGSFKVAVVASEKIKILELPYASGRLTMLVVLPDDVSGLKQLETTITFEKLMEWTTSNIMEERKIKVYLPRMKIEEKYNLTSVLMALGLTDLFSSSANLSGISSAESLKMSEAVHEAFVEIYEAGSEVVASAEAGMDATSVSEEFRADHPFLFLIKDNTSNSILFFGRCFSP

SEQ ID NO: 39 - protein, 386 aa, synthetic construct
  REGION 1..386: note = Synthetic Polypeptide
MGSIGAASTEFCFDVFKELKGQHVNENIFFCPLSIVSALSMVYLGARENTRAQIVKVAHFDKIAGFAESIESQCGTSVSIHTSLKDMFTQITKPSDNYSLNFASRLYAEETYPIIPEYLQCVKELYKGGLETISFQTAADQAREIINSWVESQTNGMIKNILRPSSVHPQTELVLVNAVYFKGTWEKAFKDEDTQAVPFRITEQESKPVQMMYQIGSFKVAAVTSEKMKILEVPYASGELSMLVLLPDDVSGLEQLETAITAEKLIEWTSSTVMEERKLKVYLPRMKIEEKYNLTTVLTALGVTDLFSSSANLSGISSAQGLKMSNAVHEAFVEIYEAGSEVVGSKGEGTEVSSVSDEFKADHPFLFLIKHNPTNSIVFFGRCFSP

SEQ ID NO: 40 - protein, 386 aa, synthetic construct
  REGION 1..386: note = Synthetic Polypeptide
MGSIGAASTEFCFDVFKELKVHHVNENILYSPLAIISALSMVYLGAKENTRDQIDKVVHFDKITGIGESIESQCSTAVSVHTSLKDVFDQITRPSDNYSLAFASRLYAEKTYPILPEYLQCVKELYKGGLETIDFQTAADQARQLINSWVEDETNGMIKNILRPSSVNPQTKIILVNAIYFKGMWEKAFKDEDTQEVPFRITEQETKSVQMMYQIGSFKVAEVVSDKMKILELPYASGKLSMLVLLPDDVYGLEQLETVITVEKLKEWTSSIVMEERITKVYLPRMKIMEKYNLTSVLTAFGITDLFSPSANLSGISSTESLKVSEAVHEAFVEIHEAGSEVVGSAGAGIEATSVSEEFKADHPFLFLIKHNPTNSILFFGRCFSP

SEQ ID NO: 41 - protein, 386 aa, synthetic construct
  REGION 1..386: note = Synthetic Polypeptide
MGSIGAASTEFCLDVFKELKVQHVNENIFYSPLSIISALSMVYLGARENTRAQIDKVVHFDKITGFEDSIESQCGTSVSVHTSLKDMFTQITKPSDNYSVGFASRLYAAETYQILPEYSQCVKELYKGGLETINFQKAADQATELINSWVESQTNGMIKNILQPSSVDPQTQIFLVNAIYFKGMWQRAFKEEDTQAVPFRISEKESKPVQMMYQIGSFKVAVIPSEKIKILELPYASGLLSMLVILPDDVSGLEQLENAITLEKLMQWTSSNMMEERKIKVYLPRMRMEEKYNLTSVFMALGITDLFSSSANLSGISSAESLKMSDAVHEASVEIHEAGSEVVGSTGSGTEASSVSEEFRADHPYLFLIKHNPTDSIVFFGRCFSP

SEQ ID NO: 42 - protein, 386 aa, synthetic construct
  REGION 1..386: note = Synthetic Polypeptide
MGSIGAASTEFCFDVFKELKFQHVDENIFYSPLTIISALSMVYLGARENTRAQIDKVVHFDKIAGFEETVESQCGTSVSVHTSLKDMFAQITKPSDNYSLSFASRLYAEETYPILPEYLQCVKELYKGGLETISFQTAADQARDLINSWVESQTNGMIKNILQPSSVGPQTELILVNAIYFKGMWQKAFKDEDTQEVPFRMTEQQSKPVQMMYQTGSFKVAVVASEKMKILALPYASGQLSLLVMLPDDVSGLKQLESAITSEKLIEWTSPSMMEERKIKVYLPRMKIEEKYNLTSVLMALGITDLFSPSANLSGISSAESLKMSQAVHEAFVEIYEAGSEVVGSTGAGMEDSSDSEEFRVDHPFLFFIKHNPTNSILFFGRCFSP

SEQ ID NO: 43 - protein, 386 aa, synthetic construct
  REGION 1..386: note = Synthetic Polypeptide
MGSIGPLSVEFCCDVFKELRIQHPRENIFYSPVTIISALSMVYLGARDNTKAQIEKAVHFDKIPGFGESIESQCGTSLSIHTSLKDIFTQITKPSDNYTVGIASRLYAEEKYPILPEYLQCIKELYKGGLEPINFQTAAEQARELINSWVESQTNGMIKNILQPSSVNPETDMVLVNAIYFKGLWEKAFKDEDIQTVPFRITEQESKPVQMMFQIGSFRVAEITSEKIRILELPYASGQLSLWVLLPDDISGLEQLETAITFENLKEWTSSTKMEERKIKVYLPRMKIEEKYNLTSVLTSLGITDLFSSSANLSGISSAESLKVSSAFHEASVEIYEAGSKVVGSTGAEVEDTSVSEEFRADHPFLFLIKHNPSNSIFFFGRCFSP

SEQ ID NO: 44 - protein, 386 aa, synthetic construct
  REGION 1..386: note = Synthetic Polypeptide
MGSIGTASAEFCFDVFKELKVHHVNENIFYSPLSIISALSMVYLGARENTKTQMEKVIHFDKITGLGESMESQCGTGVSIHTALKDMLSEITKPSDNYSLSLASRLYAEQTYAILPEYLQCIKELYKESLETVSFQTAADQARELINSWIESQTNGVIKNFLQPGSVDSQTELVLVNAIYFKGMWEKAFKDEDTQEVPFRITEQESRPVQMMYQAGSFKVATVAAEKIKILELPYASGELSMLVLLPDDISGLEQLETTISFEKLTEWTSSNMMEDRNMKVYLPRMKIEEKYNLTSVLIALGMTDLFSPAANLSGISAAESLKMSEAIHAAYVEIYEADSEIVSSAGVQVEVTSDSEEFRVDHPFLFLIKHNPTNSVLFFGRCISP

SEQ ID NO: 45 - protein, 386 aa, synthetic construct
  REGION 1..386: note = Synthetic Polypeptide
MGSIGAVSTEFSCDVFKELRIHHVQENIFYSPVTIISALSMIYLGARDSTKAQIEKAVHFDKIPGFGESIESQCGTSLSIHTSIKDMFTKITKASDNYSIGIASRLYAEEKYPILPEYLQCVKELYKGGLESISFQTAAEQAREIINSWVESQTNGMIKNILQPSSVDPQTDIVLVNAIYFKGLWEKAFRDEDTQTVPFKITEQESKPVQMMYQIGSFKVAEITSEKIKILEVPYASGQLSLWVLLPDDISGLEKLETAITFENLKEWTSSTKMEERKIKVYLPRMKIEEKYNLTSVLTALGITDLFSSSANLSGISSAESLKVSEAFHEAIVEISEAGSKVVGSVGAGVDDTSVSEEFRADHPFLFLIKHNPTSSIFFFGRCFSP

SEQ ID NO: 46 - protein, 381 aa, synthetic construct
  REGION 1..381: note = Synthetic Polypeptide
MGSIGAASTEFCFDVFKELKVQHVNENIFYSPLSIISALSMVYLGARENTRAQIDKVVHFDKIAGFGESTESQCGTSVSAHTSLKDMSNQITKLSDNYSLSFASRLYAEETYPILPEYSQCVKELYKGGLESISFQTAAYQARELINAWVESQTNGMIKDILQPGSVDSQTKMVLVNAIYFKGIWEKAFKDEDTQEVPFRMTEQETKPVQMMYQIGSFKVAVIAAEKIKILELPYASGQLSMLVILPDDVSGLEQLETAITFEKLTEWTSASVMEERKIKVYLPRMSIEEKYNLTSVLIALGVTDLFSSSANLSGISSAESLRMSEAIHEAFVETYEAGSTESGTEVTSASEEFRVDHPFLFLIKHKPTNSILFFGRCFSP

SEQ ID NO: 47 - protein, 391 aa, synthetic construct
  REGION 1..391: note = Synthetic Polypeptide
MGSIGAASSEFCFDIFKELKVQHVNENIFYSPLSIISALSMVYLGARENTRAQIDKVVPFDKITASGESIESQVQKIQCSTSVSVHTSLKDIFTQITKSSDNHSLSFASRLYAEETYPILPEYLQCVKELYEGGLETISFQTAADQARELINSWIESQTNGRIKNILQPGSVDPQTEMVLVNAIYFKGMWEKAFKDEDTQAVPFRMTEQESKPVQVMHQIGSFKVAVLASEKIKILELPYASGELSMLVLLPDDVSGLEQLETAITFEKLMEWTSPNIMEERKIKVFLPRMKIEEKYNLTSVLMALGITDLFSPLANLSGISSAESLKMSEAIHEAFVEISEAGSEVIGSTEAEVEVTNDPEEFRADHPFLFLIKHNPTNSILFFGRCFSP

SEQ ID NO: 48 - protein, 383 aa, synthetic construct
  REGION 1..383: note = Synthetic Polypeptide
MGSIGPLSVEFCCDVFKELRIQHARENIFYSPVTIISALSMVYLGARDNTKAQIEKAVHFDKIPGFGESIESQCGTSLSIHTSLKDIFTQITKPSDNYTVGIASRLYAEEKYPILPEYLQCIKELYKGGLEPISFQTAAEQARELINSWVESQTNGIIKNILQPSSVNPETDMVLVNAIYFKGLWEKAFKDEGTQTVPFRITEQESKPVQMMFQIGSFRVAEIASEKIRILELPYASGQLSLWVLLPDDISGLEQLETAITFENLKEWTSSTKMEERKIKVYLPRMKIEEKYNLTSVLTSLGITDLFSSSANLSGISSAERLKVSSAFHEASMEINEAGSKVVGAGVDDTSVSEEFRVDRPFLFLIKHNPSNSIFFFGRCFSP

SEQ ID NO: 49 - protein, 386 aa, synthetic construct
  REGION 1..386: note = Synthetic Polypeptide
MGSIGAASTEFCFDMFKELKVHHVNENIIYSPLSIISILSMVFLGARENTKTQMEKVIHFDKITGFGESLESQCGTSVSVHASLKDILSEITKPSDNYSLSLASKLYAEETYPVLPEYLQCIKELYKGSLETVSFQTAADQARELINSWVETQTNGVIKNFLQPGSVDPQTEMVLVDAIYFKGTWEKAFKDEDTQEVPFRITEQESKPVQMMYQAGSFKVATVAAEKMKILELPYASGELSMFVLLPDDISGLEQLETTISIEKLSEWTSSNMMEDRKMKVYLPHMKIEEKYNLTSVLVALGMTDLFSPSANLSGISTAQTLKMSEAIHGAYVEIYEAGSEMATSTGVLVEAASVSEEFRVDHPFLFLIKHNPSNSILFFGRCIFP

SEQ ID NO: 50 - protein, 392 aa, synthetic construct
  REGION 1..392: note = Synthetic Polypeptide
MGSIGAASTEFCFDMFKELKVHHVNENIIYSPLSIISILSMVFLGARENTKTQMEKVIHFDKITGFGESLESQCGTSVSVHASLKDILSEITKPSDNYSLSLASKLYAEETYPVLPEYLQCIKELYKGSLETVSFQTAADQARELINSWVETQTNGVIKNFLQPGSVDPQTEMVLVDAIYFKGTWEKAFKDEDTQEVPFRITEQESKPVQMMYQAGSFKVATVAAEKMKILELPYASGELSMFVLLPDDISGLEQLETTISIEKLSEWTSSNMMEDRKMKVYLPHMKIEEKYNLTSVLVALGMTDLFSPSANLSGISTAQTLKMSEAIHGAYVEIYEAGSEMATSTGVLVEAASVSEEFRVDHPFLFLIKHNPSNSILFFGRCIFPHHHHHH

SEQ ID NO: 51 - protein, 386 aa, synthetic construct
  REGION 1..386: note = Synthetic Polypeptide
MGSIGPLSVEFCCDVFKELRIQHARENIFYSPVTIISALSMVYLGARDNTKAQIEKAVHFDKIPGFGESIESQCGTSLSIHTSLKDIFTQITKPSDNYTVGIASRLYAEEKYPILPEYLQCIKELYKGGLEPISFQTAAEQARELINSWVESQTNGMIKNILQPSAVNPETDMVLVNAIYFKGLWEKAFKDEGTQTVPFRITEQESKPVQMMFQIGSFRVAEITSEKIRILELPYASGQLSLWVLLPDDISGLEQLETAITFENLKEWTSSTKMEERKIKVYLPRMKIEEKYNLTSVLTSLGITDLFSSSANLSGISSAERLKVSSAFHEASMEIYEAGSKVVGSTGAGVDDTSVSEEFRVDRPFLFLIKHNPSNSIFFFGRCFSP

SEQ ID NO: 52 - protein, 395 aa, synthetic construct
  REGION 1..395: note = Synthetic Polypeptide
  VARIANT 99: note = misc_feature - Xaa can be any naturally occurring amino acid
  VARIANT 233: note = misc_feature - Xaa can be any naturally occurring amino acid
  VARIANT 341: note = misc_feature - Xaa can be any naturally occurring amino acid
  VARIANT 379: note = misc_feature - Xaa can be any naturally occurring amino acid
MEDQRGNTGFTMGSIGAASTEFCIDVFRELRVQHVNENIFYSPLTIISALSMVYLGARENTRAQIDQVVHFDKIAGFGDTVESQCGSSPSVHNSLKTVXAQITQPRDNYSLNLASRLYAEESYPILPEYLQCVKELYNGGLETVSFQTAADQARELINSWVESQTNGIIKNILQPSSVDPQTEMVLVNAIYFKGLWEKAFKDEETQAVPFRITEQENRPVQMMYQFGSFKVAXVASEKIKILELPYASGQLSMLVLLPDEVSGLEQNAITFEKLTEWTSSDLMEERKIKVFFPRVKIEEKYNLTAVLVSLGITDLFSSSANLSGISSAENLKMSEAVHEAXVEIYEAGSEVAGSSGAGIEVASDSEEFRVDHPFLFLIXHNPTNSILFFGRCFSP

SEQ ID NO: 53 - protein, 386 aa, synthetic construct
  REGION 1..386: note = Synthetic Polypeptide
MGSIGAASTEFCIDVFRELRVQHVNENIFYSPLSIISALSMVYLGARENTRAQIDEVFHFDKIAGFGDTVDPQCGASLSVHKSLQNVFAQITQPKDNYSLNLASRLYAEESYPILPEYLQCVKELYNEGLETVSFQTGADQARELINSWVENQTNGVIKNILQPSSVDPQTEMVLVNAIYFKGLWQKAFKDEETQAVPFRITEQENRPVQMMYQFGSFKVAVVASEKVKILELPYASGQLSMWVLLPDEVSGLEQLENAITFEKLTEWTSSDLTEERKIKVFLPRVKIEEKYNLTAVLMALGVTDLFSSSANFSGISAAENLKMSEAVHEAFVEIYEAGSEVVGSSGAGIEAPSDSEEFRADHPFLFLIKHNPTNSILFFGRCFSP

SEQ ID NO: 54 - protein, 386 aa, synthetic construct
  REGION 1..386: note = Synthetic Polypeptide
MGSIGPLSVEFCCDVFKELRIQHARDNIFYSPVTIISALSMVYLGARDNTKAQIEKAVHFDKIPGFGESIESQCGTSLSVHTSLKDIFTQITKPRENYTVGIASRLYAEEKYPILPEYLQCIKELYKGGLEPISFQTAAEQARELINSWVESQTNGMIKNILQPSSVNPETDMVLVNAIYFKGLWKKAFKDEGTQTVPFRITEQESKPVQMMFQIGSFRVAEITSEKIRILELPYASGQLSLWVLLPDDISGLEQLESAITFENLKEWTSSTKMEERKIKVYLPRMKIEEKYNLTSVLTSLGITDLFSSSANLSGISSAEKLKVSSAFHEASMEIYEAGNKVVGSTGAGVDDTSVSEEFRVDRPFLFLIKHNPSNSIFFFGRCFSP

SEQ ID NO: 55 - protein, 385 aa, synthetic construct
  REGION 1..385: note = Synthetic Polypeptide
MGSIGAASAEFCVDVFKELKDQHVNNIVFSPLMIISALSMVNIGAREDTRAQIDKVVHFDKITGYGESIESQCGTSIGIYFSLKDAFTQITKPSDNYSLSFASKLYAEETYPILPEYLKCVKELYKGGLETISFQTAADQARELINSWVESQTNGMIKNILQPSSVDPQTEMVLVNAIYFKGLWEKAFKDEDTQAVPFRITEQESKPVQMMYQIGSFKVAVIASEKIKILELPYASGQLSLLVLLPDDVSGLEQLESAITSEKLLEWTNPNIMEERKTKVYLPRMKIEEKYNLTSVLVALGITDLFSSSANLSGISSAEGLKLSDAVHEAFVEIYEAGREVVGSSEAGVEDSSVSEEFKADRPFIFLIKHNPTNGILYFGRYISP

SEQ ID NO: 56 - protein, 386 aa, synthetic construct
  REGION 1..386: note = Synthetic Polypeptide
MGSIGAANTDFCFDVFKELKVHHANENIFYSPLSIVSALAMVYLGARENTRAQIDKALHFDKILGFGETVESQCDTSVSVHTSLKDMLIQITKPSDNYSFSFASKIYTEETYPILPEYLQCVKELYKGGVETISFQTAADQAREVINSWVESHTNGMIKNILQPGSVDPQTKMVLVNAVYFKGIWEKAFKEEDTQEMPFRINEQESKPVQMMYQIGSFKLTVAASENLKILEFPYASGQLSMMVILPDEVSGLKQLETSITSEKLIKWTSSNTMEERKIRVYLPRMKIEEKYNLKSVLMALGITDLFSSSANLSGISSAESLKMSEAVHEAFVEIYEAGSEVTSSTGTEMEAENVSEEFKADHPFLFLIKHNPTDSIVFFGRCMSP

SEQ ID NO: 57 - protein, 383 aa, synthetic construct
  REGION 1..383: note = Synthetic Polypeptide
MGSIGPLSVEFCCDVFKELRIQHARENIFYSPVTIISALSMVYLGARDNTKAQIEKAVHFDKIPGFGESIESQCGTSLSIHTSLKDIFTQITKPSDNYTVGIASRLYAEEKYPILPEYLQCIKELYKGGLEPISFQTAAEQARELINSWVESQTNGMIKNILQPSSVNPETDMVLVNAIYFKGLWEKAFKDESTQTVPFRITEQESKPVQMMFQIGSFRVAEIASEKIRILELPYASGQLSLWVLLPDDISGLEQLETAITFENLKEWTSSTKMEERKIKVYLPRMKIEEKYNLTSVLTSLGITDLFSSSANLSGISSAERLKVSSAFHEASMEIYEAGSRVVEAGVDDTSVSEEFRVDRPFLFLIKHNPSNSIFFFGRCFSP

SEQ ID NO: 58 - protein, 386 aa, synthetic construct
  REGION 1..386: note = Synthetic Polypeptide
MGSIGPVSTEFCCDIFKELRIQHARENIIYSPVTIISALSMVYLGARDNTKAQIEKAVHFDKIPGFGESIESQCGTSLSIHTSLKDILTQITKPSDNYTVGIASRLYAEEKYPILSEYLQCIKELYKGGLEPISFQTAAEQARELINSWVESQTNGMIKNILQPSSVNPETDMVLVNAIYFKGLWEKAFKDEGTQTVPFRITEQESKPVQMMFQIGSFKVAEITSEKIRILELPYASGKLSLWVLLPDDISGLEQLETAITFENLKEWTSSTRMEERKIKVYLPRMKIEEKYNLTSVLTSLGITDLFSSSANLSGISSAERLKVSSAFHEVFVEIYEAGSKVEGSTGAGVDDTSVSEEFRADHPFLFLVKHNPSNSIIFFGRCYLP

SEQ ID NO: 59 - protein, 386 aa, synthetic construct
  REGION 1..386: note = Synthetic Polypeptide
MGSTGAASMEFCFALFRELKVQHVNENIFFSPVTIISALSMVYLGARENTRAQLDKVAPFDKITGFGETIGSQCSTSASSHTSLKDVFTQITKASDNYSLSFASRLYAEETYPILPEYLQCVKELYKGGLESISFQTAADQARELINSWVESQTNGMIKDILRPSSVDPQTKIILITAIYFKGMWEKAFKEEDTQAVPFRMTEQESKPVQMMYQIGSFKVAVIPSEKLKILELPYASGQLSMLVILPDDVSGLEQLETAITTEKLKEWTSPSMMKERKMKVYFPRMRIEEKYNLTSVLMALGITDLFSPSANLSGISSAESLKVSEAVHEASVDIDEAGSEVIGSTGVGTEVTSVSEEIRADHPFLFLIKHKPTNSILFFGRCFSP

SEQ ID NO: 60 - protein, 2174 aa, synthetic construct
  REGION 1..2174: note = Synthetic Polypeptide
MEHAQLTQLVNSNMTSNTCHEADEFENIDFRMDSISVTNTKFCFDVFNEMKVHHVNENILYSPLSILTALAMVYLGARGNTESQMKKALHFDSITGAGSTTDSQCGSSEYIHNLFKEFLTEITRTNATYSLEIADKLYVDKTFTVLPEYINCARKFYTGGVEEVNFKTAAEEARQLINSWVEKETNGQIKDLLVPSSVDFGTMMVFINTIYFKGIWKTAFNTEDTREMPFSMTKQESKPVQMMCLNDTFNMATLPAEKMRILELPYASGELSMLVLLPDEVSGLEQIEKAINFEKLREWTSTNAMEKKSMKVYLPRMKIEEKYNLTSTLMALGMTDLFSRSANLTGISSVENLMISDAVHGAFMEVNEEGTEAAGSTGAIGNIKHSVEFEEFRADHPFLFLIRYNPTNVILFFDNSEFTMGSIGAVSTEFCFDVFKELRVHHANENIFYSPFTVISALAMVYLGAKDSTRTQINKVVRFDKLPGFGDSIEAQCGTSANVHSSLRDILNQITKPNDIYSFSLASRLYADETYTILPEYLQCVKELYRGGLESINFQTAADQARELINSWVESQTSGIIRNVLQPSSVDSQTAMVLVNAIYFKGLWEKGFKDEDTQAMPFRVTEQENKSVQMMYQIGTFKVASVASEKMKILELPFASGTMSMWVLLPDEVSGLEQLETTISIEKLTEWTSSSVMEERKIKVFLPRMKMEEKYNLTSVLMAMGMTDLFSSSANLSGISSTLQKKGFRSQELGDKYAKPMLESPALTPQVTAWDNSWIVAHPAAIEPDLCYQIMEQKWKPFDWPDFRLPMRVSCRFRTMEALNKANTSFALDFFKHECQEDDDENILFSPFSISSALATVYLGAKGNTADQMAKTEIGKSGNIHAGFKALDLEINQPTKNYLLNSVNQLYGEKSLPFSKEYLQLAKKYYSAEPQSVDFLGKANEIRREINSRVEHQTEGKIKNLLPPGSIDSLTRLVLVNALYFKGNWATKFEAEDTRHRPFRINMHTTKQVPMMYLRDKFNWTYVESVQTDVLELPYVNNDLSMFILLPRDITGLQKLINELTFEKLSAWTSPELMEKMKMEVYLPRFTVEKKYDMKSTLSKMGIEDAFTKVDSCGVTNVDEITTHIVSSKCLELKHIQINKKLKCNKAVAMEQVSASIGNFTIDLFNKLNETSRDKNIFFSPWSVSSALALTSLAAKGNTAREMAEDPENEQAENIHSGFKELMTALNKPRNTYSLKSANRIYVEKNYPLLPTYIQLSKKYYKAEPYKVNFKTAPEQSRKEINNWVEKQTERKIKNFLSSDDVKNSTKSILVNAIYFKAEWEEKFQAGNTDMQPFRMSKNKSKLVKMMYMRHTFPVLIMEKLNFKMIELPYVKRELSMFILLPDDIKDSTTGLEQLERELTYEKLSEWADSKKMSVTLVDLHLPKFSMEDRYDLKDALKSMGMASAFNSNADFSGMTGFQAVPMESLSASTNSFTLDLYKKLDETSKGQNIFFASWSIATALAMVHLGAKGDTATQVAKGPEYEETENIHSGFKELLSAINKPRNTYLMKSANRLFGDKTYPLLPKFLELVARYYQAKPQAVNFKTDAEQARAQINSWVENETESKIQNLLPAGSIDSHTVLVLVNAIYFKGNWEKRFLEKDTSKMPFRLSKTETKPVQMMFLKDTFLIHHERTMKFKIIELPYVGNELSAFVLLPDDISDNTTGLELVERELTYEKLAEWSNSASMMKAKVELYLPKLKMEENYDLKSVLSDMGIRSAFDPAQADFTRMSEKKDLFISKVIHKAFVEVNEEDRIVQLASGRLTGRCRTLANKELSEKNRTKNLFFSPFSISSALSMILLGSKGNTEAQIAKVLSLSKAEDAHNGYQSLLSEINNPDTKYILRTANRLYGEKTFEFLSSFIDSSQKFYHAGLEQTDFKNASEDSRKQINGWVEEKTEGKIQKLLSEGIINSMTKLVLVNAIYFKGNWQEKFDKETTKEMPFKINKNETKPVQMMFRKGKYNMTYIGDLETTVLEIPYVDNELSMIILLPDSIQDESTGLEKLERELTYEKLMDWINPNMMDSTEVRVSLPRFKLEENYELKPTLSTMGMPDAFDLRTADFSGISSGNELVLSEVVHKSFVEVNEEGTEAAAATAGIMLLRCAMIVANFTADHPFLFFIRHNKTNSILFCGRFCSP

SEQ ID NO: 61 - protein, 386 aa, synthetic construct
  REGION 1..386: note = Synthetic Polypeptide
MGSIGTASTEFCFDMFKEMKVQHANQNIIFSPLTIISALSMVYLGARDNTKAQMEKVIHFDKITGFGESVESQCGTSVSIHTSLKDMLSEITKPSDNYSLSLASRLYAEETYPILPEYLQCMKELYKGGLETVSFQTAADQARELINSWVESQTNGVIKNFLQPGSVDPQTEMVLVNAIYFKGMWEKAFKDEDTQEVPFRITEQESKPVQMMYQVGSFKVATVAAEKMKILEIPYTHRELSMFVLLPDDISGLEQLETTISFEKLTEWTSSNMMEERKVKVYLPHMKIEEKYNLTSVLMALGMTDLFSPSANLSGISTAQTLMMSEAIHGAYVEIYEAGREMASSTGVQVEVTSVLEEVRADKPFLFFIRHNPTNSMVVFGRYMSP

SEQ ID NO: 62 - protein, 2104 aa, synthetic construct
  REGION 1..2104: note = Synthetic Polypeptide
MTSNTCHEADEFENIDFRMDSISVTNTKFCFDVFNEMKVHHVNENILYSPLSILTALAMVYLGARGNTESQMKKALHFDSITGGGSTTDSQCGSSEYIHNLFKEFLTEITRTNATYSLEIADKLYVDKTFTVLPEYINCARKFYTGGVEEVNFKTAAEEARQLMNSWVEKETNGQIKDLLVPSSVDFGTMMVFINTIYFKGIWKTAFNTEDTREMPFSMTKQESKPVQMMCLNDTFNMVTLPAEKMRILELPYASGELSMLVLLPDEVSGLERIEKAINFEKLREWTSTNAMEKKSMKVYLPRMKIEEKYNLTSTLMALGMTDLFSRSANLTGISSVDNLMISDAVHGAFMEVNEEGTEAAGSTGAIGNIKHSVEFEEFRADHPFLFLIRYNPTNVILFFDNSEFTMGSIGAVSTEFCFDVFKELRVHHANENIFYSPFTIISALAMVYLGAKDSTRTQINKVVRFDKLPGFGDSIEAQCGTSANVHSSLRDILNQITKPNDIYSFSLASRLYADETYTILPEYLQCVKELYRGGLESINFQTAADQARELINSWVESQTSGIIRNVLQPSSVDSQTAMVLVNAIYFKGLWEKGFKDEDTQAIPFRVTEQENKSVQMMYQIGTFKVASVASEKMKILELPFASGTMSMWVLLPDEVSGLEQLETTISIEKLTEWTSSSVMEERKIKVFLPRMKMEEKYNLTSVLMAMGMTDLFSSSANLSGISSTLQKKGFRSQELGDKYAKPMLESPALTPQATAWDNSWIVAHPPAIEPDLYYQIMEQKWKPFDWPDFRLPMRVSCRFRTMEALNKANTSFALDFFKHECQEDDSENILFSPFSISSALATVYLGAKGNTADQMAKVLHFNEAEGARNVTTTIRMQVYSRTDQQRLNRRACFQKTEIGKSGNIHAGFKGLNLEINQPTKNYLLNSVNQLYGEKSLPFSKEYLQLAKKYYSAEPQSVDFVGTANEIRREINSRVEHQTEGKIKNLLPPGSIDSLTRLVLVNALYFKGNWATKFEAEDTRHRPFRINTHTTKQVPMMYLSDKFNWTYVESVQTDVLELPYVNNDLSMFILLPRDITGLQKLINELTFEKLSAWTSPELMEKMKMEVYLPRFTVEKKYDMKSTLSKMGIEDAFTKVDNCGVTNVDEITIHVVPSKCLELKHIQINKELKCNKAVAMEQVSASIGNFTIDLFNKLNETSRDKNIFFSPWSVSSALALTSLAAKGNTAREMAEDPENEQAENIHSGFNELLTALNKPRNTYSLKSANRIYVEKNYPLLPTYIQLSKKYYKAEPHKVNFKTAPEQSRKEINNWVEKQTERKIKNFLSSDDVKNSTKLILVNAIYFKAEWEEKFQAGNTDMQPFRMSKNKSKLVKMMYMRHTFPVLIMEKLNFKMIELPYVKRELSMFILLPDDIKDSTTGLEQLERELTYEKLSEWADSKKMSVTLVDLHLPKFSMEDRYDLKDALRSMGMASAFNSNADFSGMTGERDLVISKVCHQSFVAVDEKGTEAAAATAVIAEAVPMESLSASTNSFTLDLYKKLDETSKGQNIFFASWSIATALTMVHLGAKGDTATQVAKGPEYEETENIHSGFKELLSALNKPRNTYSMKSANRLFGDKTYPLLPTKTKPVQMMFLKDTFLIHHERTMKFKIIELPYMGNELSAFVLLPDDISDNTTGLELVERELTYEKLAEWSNSASMMKVKVELYLPKLKMEENYDLKSALSDMGIRSAFDPAQADFTRMSEKKDLFISKVIHKAFVEVNEEDRIVQLASGRLTGNTEAQIAKVLSLSKAEDAHNGYQSLLSEINNPDTKYILRTANRLYGEKTFEFLSSFIDSSQKFYHAGLEQTDFKNASEDSRKQINGWVEEKTEGKIQKLLSEGIINSMTKLVLVNAIYFKGNWQEKFDKETTKEMPFKINKNETKPVQMMFRKGKYNMTYIGDLETTVLEIPYVDNELSMIILLPDSIQDESTGLEKLERELTYEKLMDWINPNMMDSTEVRVSLPRFKLEENYELKPTLSTMGMPDAFDLRTADFSGISSGNELVLSEVVHKSFVEVNEEGTEAAAATAGIMLLRCAMIVANFTADHPFLFFIRHNKTNSILFCGRFCSP

SEQ ID NO: 63 - protein, 386 aa, synthetic construct
  REGION 1..386: note = Synthetic Polypeptide
MASIGAASTEFCFDVFKELKTQHVKENIFYSPMAIISALSMVYIGARENTRAEIDKVVHFDKITGFGNAVESQCGPSVSVHSSLKDLITQISKRSDNYSLSYASRIYAEETYPILPEYLQCVKEVYKGGLESISFQTAADQARENINAWVESQTNGMIKNILQPSSVNPQTEMVLVNAIYLKGMWEKAFKDEDTQTMPFRVTQQESKPVQMMYQIGSFKVAVIASEKMKILELPYTSGQLSMLVLLPDDVSGLEQVESAITAEKLMEWTSPSIMEERTMKVYLPRMKMVEKYNLTSVLMALGMTDLFTSVANLSGISSAQGLKMSQAIHEAFVEIYEAGSEAVGSTGVGMEITSVSEEFKADLSFLFLIRHNPTNSIIFFGRCISP

SEQ ID NO: 64 - protein, 420 aa, synthetic construct
  REGION 1..420: note = Synthetic Polypeptide
MGSIGAASTEFCFDVFRELRVQHVNENIFYSPFSIISALAMVYLGARDNTRTQIDKISQFQALSDEHLVLCIQQLGEFFVCTNRERREVTRYSEQTEDKTQDQNTGQIHKIVDTCMLRQDILTQITKPSDNFSLSFASRLYAEETYAILPEYLQCVKELYKGGLESISFQTAADQARELINSWVESQTNGIIKNILQPSSVDSQTTMVLVNAIYFKGMWEKAFKDEDTQAMPFRMTEQESKPVQMMYQVGSFKVAMVTSEKMKILELPFASGMMSMFVLLPDEVSGLEQLESTISFEKLTEWTSSTMMEERRMKVYLPRMKMEEKYNLTSVFMALGMTDLFSSSANMSGISSTVSLKMSEAVHAACVEIFEAGRDVVGSAEAGMDVTSVSEEFRADHPFLFFIKHNPTNSILFFGRWMSP

SEQ ID NO: 65 - protein, 386 aa, synthetic construct
  REGION 1..386: note = Synthetic Polypeptide
MGSIGAASAEFCLDIFKELKVQHVNENIIFSPMTIISALSLVYLGAKEDTRAQIEKVVPFDKIPGFGEIVESQCPKSASVHSSIQDIFNQIIKRSDNYSLSLASRLYAEESYPIRPEYLQCVKELDKEGLETISFQTAADQARQLINSWVESQTNGMIKNILQPSSVNSQTEMVLVNAIYFRGLWQKAFKDEDTQAVPFRITEQESKPVQMMQQIGSFKVAEIASEKMKILELPYASGQLSMLVLLPDDVSGLEKLESSITVEKLIEWTSSNLTEERNVKVYLPRLKIEEKYNLTSVLAALGITDLFSSSANLSGISTAESLKLSRAVHESFVEIQEAGHEVEGPKEAGIEVTSALDEFRVDRPFLFVTKHNPTNSILFLGRCLSP

SEQ ID NO: 66 - protein, 386 aa, synthetic construct
  REGION 1..386: note = Synthetic Polypeptide
MGSISAASGEFCLDIFKELKVQHVNENIFYSPMVIVSALSLVYLGARENTRAQIDKVIPFDKITGSSEAVESQCGTPVGAHISLKDVFAQIAKRSDNYSLSFVNRLYAEETYPILPEYLQCVKELYKGGLETISFQTAADQAREIINSWVESQTDGKIKNILQPSSVDPQTKMVLVSAIYFKGLWEKSFKDEDTQAVPFRVTEQESKPVQMMYQIGSFKVAAIAAEKIKILELPYASEQLSMLVLLPDDVSGLEQLEKKISYEKLTEWTSSSVMEEKKIKVYLPRMKIEEKYNLTSILMSLGITDLFSSSANLSGISSTKSLKMSEAVHEASVEIYEAGSEASGITGDGMEATSVFGEFKVDHPFLFMIKHKPTNSILFFGRCISP

SEQ ID NO: 67 - protein, 386 aa, synthetic construct
  REGION 1..386: note = Synthetic Polypeptide
MGSIGPVSTEVCCDIFRELRSQSVQENVCYSPLLIISTLSMVYIGAKDNTKAQIEKAIHFDKIPGFGESTESQCGTSVSIHTSLKDIFTQITKPSDNYSISIARRLYAEEKYPILPEYIQCVKELYKGGLESISFQTAAEKSRELINSWVESQTNGTIKNILQPSSVSSQTDMVLVSAIYFKGLWEKAFKEEDTQTIPFRITEQESKPVQMMSQIGTFKVAEIPSEKCRILELPYASGRLSLWVLLPDDISGLEQLETAITFENLKEWTSSSKMEERKIRVYLPRMKIEEKYNLTSVLKSLGITDLFSSSANLSGISSAESLKVSAAFHEASVEIYEAGSKGVGSSEAGVDGTSVSEEIRADHPFLFLIKHNPSDSILFFGRCFSP

SEQ ID NO: 68 - protein, 386 aa, synthetic construct
  REGION 1..386: note = Synthetic Polypeptide
MGSIGAASTEFCFDVFKELKVQHVNENIIISPLSIISALSMVYLGAREDTRAQIDKVVHFDKITGFGEAIESQCPTSESVHASLKETFSQLTKPSDNYSLAFASRLYAEETYPILPEYLQCVKELYKGGLETINFQTAAEQARQVINSWVESQTDGMIKSLLQPSSVDPQTEMILVNAIYFRGLWERAFKDEDTQELPFRITEQESKPVQMMSQIGSFKVAVVASEKVKILELPYASGQLSMLVLLPDDVSGLEQLESSITVEKLIEWISSNTKEERNIKVYLPRMKIEEKYNLTSVLVALGITDLFSSSANLSGISSAESLKISEAVHEAFVEIQEAGSEVVGSPGPEVEVTSVSEEWKADRPFLFLIKHNPTNSILFFGRYISP

SEQ ID NO: 69 - protein, 386 aa, synthetic construct
  REGION 1..386: note = Synthetic Polypeptide
MGSIGPVSTEVCCDIFRELRSQSVQENVCYSPLLIISTLSMVYIGAKDNTKAQIEKAIHFDKIPGFGESTESQCGTSVSIHTSLKDIFTQITKPSDNYSISIARRLYAEEKYPILQEYIQCVKELYKGGLESISFQTAAEKSRELINSWVESQTNGTIKNILQPSSVSSQTDMVLVSAIYFKGLWEKAFKEEDTQTIPFRITEQESKPVQMMSQIGTFKVAEIPSEKCRILELPYASGRLSLWVLLPDDISGLEQLETSITFENLKEWTSSSKMEERKIRVYLPRMKIEEKYNLTSVLKSLGITDLFSSSANLSGISSAESLKVSAVFHEASVEIYEAGSKGVGSSEAGVDGTSVSEEIRADHPFLFLIKHNPSDSILFFGRCFSP

SEQ ID NO: 70 - protein, 399 aa, synthetic construct
  REGION 1..399: note = Synthetic Polypeptide
MLNLMHPKQFCCTMGSIGPVSTEVCCDIFRELRSQSVQENVCYSPLLIISTLSMVYIGAKDNTKAQIEKAIHFDKIPGFGESTESQCGTSVSIHTSLKDIFTQITKPSDNYSISIASRLYAEEKYPILPEYIQCVKELYKGGLESISFQTAAEKSRELINSWVESQTNGTIKNILQPSSVSSQTDMVLVSAIYFKGLWEKAFKEEDTQTVPFRITEQESKPVQMMSQIGTFKVAEIPSEKCRILELPYASGRLSLWVLLPDDISGLEQLETAITSENLKEWTSSSKMEERKIKVYLPRMKIEEKYNLTSVLKSLGITDLFSSSANLSGISSAESLKVSGAFHEAFVEIYEAGSKAVGSSGAGVEDTSVSEEIRADHPFLFFIKHNPSDSILFFGRCFSP

SEQ ID NO: 71 - protein, 389 aa, synthetic construct
  REGION 1..389: note = Synthetic Polypeptide
EAEAGSIGTASAEFCFDVFKELKVHHVNENIFYSPLSIISALSMVYLGARENTKTQMEKVIHFDKITGLGESMESQCGTGVSIHTALKDMLSEITKPSDNYSLSLASRLYAEQTYAILPEYLQCIKELYKESLETVSFQTAADQARELINSWIESQTNGVIKNFLQPGSVDSQTELVLVNAIYFKGMWEKAFKDEDTQEVPFRITEQESRPVQMMYQAGSFKVATVAAEKIKILELPYASGELSMLVLLPDDISGLEQLETTISFEKLTEWTSSNMMEDRNMKVYLPRMKIEEKYNLTSVLIALGMTDLFSPAANLSGISAAESLKMSEAIHAAYVEIYEADSEIVSSAGVQVEVTSDSEEFRVDHPFLFLIKHNPTNSVLFFGRCISP

SEQ ID NO: 72 - protein, 474 aa, synthetic construct
  REGION 1..474: note = Synthetic Polypeptide
MRFPSIFTAVLFAASSALAAPVNTTTEDETAQIPAEAVIGYSDLEGDFDVAVLPFSNSTNNGLLFINTTIASIAAKEEGVSLEKREAEAGSIGTASAEFCFDVFKELKVHHVNENIFYSPLSIISALSMVYLGARENTKTQMEKVIHFDKITGLGESMESQCGTGVSIHTALKDMLSEITKPSDNYSLSLASRLYAEQTYAILPEYLQCIKELYKESLETVSFQTAADQARELINSWIESQTNGVIKNFLQPGSVDSQTELVLVNAIYFKGMWEKAFKDEDTQEVPFRITEQESRPVQMMYQAGSFKVATVAAEKIKILELPYASGELSMLVLLPDDISGLEQLETTISFEKLTEWTSSNMMEDRNMKVYLPRMKIEEKYNLTSVLIALGMTDLFSPAANLSGISAAESLKMSEAIHAAYVEIYEADSEIVSSAGVQVEVTSDSEEFRVDHPFLFLIKHNPTNSVLFFGRCISP

SEQ ID NO: 73 - protein, 389 aa, synthetic construct
  REGION 1..389: note = Synthetic Polypeptide
EAEAGSIGAASTEFCFDVFRELRVQHVNENIFYSPFSIISALAMVYLGARDNTRTQIDKVVHFDKLPGFGESMEAQCGTSVSVHSSLRDILTQITKPSDNFSLSFASRLYAEETYAILPEYLQCVKELYKGGLESISFQTAADQARELINSWVESQTNGIIKNILQPSSVDSQTTMVLVNAIYFKGMWEKAFKDEDTQAMPFRMTEQESKPVQMMYQVGSFKVAMVTSEKMKILELPFASGMMSMFVLLPDEVSGLEQLESTISFEKLTEWTSSTMMEERRMKVYLPRMKMEEKYNLTSVFMALGMTDLFSSSANMSGISSTVSLKMSEAVHAACVEIFEAGRDVVGSAEAGMDVTSVSEEFRADHPFLFFIKHNPTNSILFFGRWMSP

SEQ ID NO: 74 - protein, 474 aa, synthetic construct
  REGION 1..474: note = Synthetic Polypeptide
MRFPSIFTAVLFAASSALAAPVNTTTEDETAQIPAEAVIGYSDLEGDFDVAVLPFSNSTNNGLLFINTTIASIAAKEEGVSLEKREAEAGSIGAASTEFCFDVFRELRVQHVNENIFYSPFSIISALAMVYLGARDNTRTQIDKVVHFDKLPGFGESMEAQCGTSVSVHSSLRDILTQITKPSDNFSLSFASRLYAEETYAILPEYLQCVKELYKGGLESISFQTAADQARELINSWVESQTNGIIKNILQPSSVDSQTTMVLVNAIYFKGMWEKAFKDEDTQAMPFRMTEQESKPVQMMYQVGSFKVAMVTSEKMKILELPFASGMMSMFVLLPDEVSGLEQLESTISFEKLTEWTSSTMMEERRMKVYLPRMKMEEKYNLTSVFMALGMTDLFSSSANMSGISSTVSLKMSEAVHAACVEIFEAGRDVVGSAEAGMDVTSVSEEFRADHPFLFFIKHNPTNSILFFGRWMSP

SEQ ID NO: 75 - protein, 4 aa, synthetic construct
  REGION 1..4: note = Synthetic Polypeptide
EAEA